European Patent Application EP 4 155 404 A1, published March 29, 2023. Title: Blood-brain barrier penetration aptamer and use thereof. Applicant: Aptamer Sciences Inc. The sequence listing filed with the application follows.

SEQUENCE LISTING (52 sequences)

SEQ ID NO: 1 - DNA, 41 bp, Artificial Sequence
  TfR-01-01-41
  misc_feature (4): B is Bn-dU.
  misc_feature (5): B is Bn-dU.
  misc_feature (12): B is Bn-dU.
  misc_feature (14): B is Bn-dU.
  misc_feature (18): B is Bn-dU.
  misc_feature (21): B is Bn-dU.
  misc_feature (22): B is Bn-dU.
  misc_feature (23): B is Bn-dU.
  misc_feature (27): B is Bn-dU.
  misc_feature (30): B is Bn-dU.
  misc_feature (34): B is Bn-dU.
  misc_feature (39): B is Bn-dU.
  misc_feature (41): B is Bn-dU.
gaabbcaaaagbgbcggbgabbbgccbcgbcgcbccaabgb

SEQ ID NO: 2 - DNA, 34 bp, Artificial Sequence
  TfR-01-01-34
  misc_feature (4): B is Bn-dU.
  misc_feature (5): B is Bn-dU.
  misc_feature (12): B is Bn-dU.
  misc_feature (14): B is Bn-dU.
  misc_feature (18): B is Bn-dU.
  misc_feature (21): B is Bn-dU.
  misc_feature (22): B is Bn-dU.
  misc_feature (23): B is Bn-dU.
  misc_feature (27): B is Bn-dU.
  misc_feature (30): B is Bn-dU.
  misc_feature (34): B is Bn-dU.
gaabbcaaaagbgbcggbgabbbgccbcgbcgcb

SEQ ID NO: 3 - DNA, 32 bp, Artificial Sequence
  TfR-01-01-32
  misc_feature (3): B is Bn-dU.
  misc_feature (5): B is Bn-dU.
  misc_feature (9): B is Bn-dU.
  misc_feature (12): B is Bn-dU.
  misc_feature (13): B is Bn-dU.
  misc_feature (14): B is Bn-dU.
  misc_feature (18): B is Bn-dU.
  misc_feature (21): B is Bn-dU.
  misc_feature (25): B is Bn-dU.
  misc_feature (30): B is Bn-dU.
  misc_feature (32): B is Bn-dU.
agbgbcggbgabbbgccbcgbcgcbccaabgb

SEQ ID NO: 4 - DNA, 26 bp, Artificial Sequence
  TfR-01-01-26
  misc_feature (4): B is Bn-dU.
  misc_feature (6): B is Bn-dU.
  misc_feature (10): B is Bn-dU.
  misc_feature (13): B is Bn-dU.
  misc_feature (14): B is Bn-dU.
  misc_feature (15): B is Bn-dU.
  misc_feature (19): B is Bn-dU.
  misc_feature (22): B is Bn-dU.
  misc_feature (26): B is Bn-dU.
aagbgbcggbgabbbgccbcgbcgcb

SEQ ID NO: 5 - DNA, 41 bp, Artificial Sequence; identical to SEQ ID NO: 1
  AMe 1
  misc_feature (2): A is a base in which the -OH group at the 2nd carbon position in the nucleotide is substituted with methoxy.
  misc_feature (4): B is Bn-dU.
  misc_feature (5): B is Bn-dU.
  misc_feature (12): B is Bn-dU.
  misc_feature (14): B is Bn-dU.
  misc_feature (18): B is Bn-dU.
  misc_feature (21): B is Bn-dU.
  misc_feature (22): B is Bn-dU.
  misc_feature (23): B is Bn-dU.
  misc_feature (27): B is Bn-dU.
  misc_feature (30): B is Bn-dU.
  misc_feature (34): B is Bn-dU.
  misc_feature (39): B is Bn-dU.
  misc_feature (41): B is Bn-dU.

SEQ ID NO: 6 - DNA, 41 bp, Artificial Sequence; identical to SEQ ID NO: 1
  AMe 2
  misc_feature (3): A is a base in which the -OH group at the 2nd carbon position in the nucleotide is substituted with methoxy.
  misc_feature (4): B is Bn-dU.
  misc_feature (5): B is Bn-dU.
  misc_feature (12): B is Bn-dU.
  misc_feature (14): B is Bn-dU.
  misc_feature (18): B is Bn-dU.
  misc_feature (21): B is Bn-dU.
  misc_feature (22): B is Bn-dU.
  misc_feature (23): B is Bn-dU.
  misc_feature (27): B is Bn-dU.
  misc_feature (30): B is Bn-dU.
  misc_feature (34): B is Bn-dU.
  misc_feature (39): B is Bn-dU.
  misc_feature (41): B is Bn-dU.

SEQ ID NO: 7 - DNA, 41 bp, Artificial Sequence; identical to SEQ ID NO: 1
  AMe 3
  misc_feature (4): B is Bn-dU.
  misc_feature (5): B is Bn-dU.
  misc_feature (7): A is a base in which the -OH group at the 2nd carbon position in the nucleotide is substituted with methoxy.
  misc_feature (12): B is Bn-dU.
  misc_feature (14): B is Bn-dU.
  misc_feature (18): B is Bn-dU.
  misc_feature (21): B is Bn-dU.
  misc_feature (22): B is Bn-dU.
  misc_feature (23): B is Bn-dU.
  misc_feature (27): B is Bn-dU.
  misc_feature (30): B is Bn-dU.
  misc_feature (34): B is Bn-dU.
  misc_feature (39): B is Bn-dU.
  misc_feature (41): B is Bn-dU.

SEQ ID NO: 8 - DNA, 41 bp, Artificial Sequence; identical to SEQ ID NO: 1
  AMe 4
  misc_feature (4): B is Bn-dU.
  misc_feature (5): B is Bn-dU.
  misc_feature (8): A is a base in which the -OH group at the 2nd carbon position in the nucleotide is substituted with methoxy.
  misc_feature (12): B is Bn-dU.
  misc_feature (14): B is Bn-dU.
  misc_feature (18): B is Bn-dU.
  misc_feature (21): B is Bn-dU.
  misc_feature (22): B is Bn-dU.
  misc_feature (23): B is Bn-dU.
  misc_feature (27): B is Bn-dU.
  misc_feature (30): B is Bn-dU.
  misc_feature (34): B is Bn-dU.
  misc_feature (39): B is Bn-dU.
  misc_feature (41): B is Bn-dU.

SEQ ID NO: 9 - DNA, 41 bp, Artificial Sequence; identical to SEQ ID NO: 1
  AMe 5
  misc_feature (4): B is Bn-dU.
  misc_feature (5): B is Bn-dU.
  misc_feature (9): A is a base in which the -OH group at the 2nd carbon position in the nucleotide is substituted with methoxy.
  misc_feature (12): B is Bn-dU.
  misc_feature (14): B is Bn-dU.
  misc_feature (18): B is Bn-dU.
  misc_feature (21): B is Bn-dU.
  misc_feature (22): B is Bn-dU.
  misc_feature (23): B is Bn-dU.
  misc_feature (27): B is Bn-dU.
  misc_feature (30): B is Bn-dU.
  misc_feature (34): B is Bn-dU.
  misc_feature (39): B is Bn-dU.
  misc_feature (41): B is Bn-dU.

SEQ ID NO: 10 - DNA, 41 bp, Artificial Sequence; identical to SEQ ID NO: 1
  AMe 6
  misc_feature (4): B is Bn-dU.
  misc_feature (5): B is Bn-dU.
  misc_feature (10): A is a base in which the -OH group at the 2nd carbon position in the nucleotide is substituted with methoxy.
  misc_feature (12): B is Bn-dU.
  misc_feature (14): B is Bn-dU.
  misc_feature (18): B is Bn-dU.
  misc_feature (21): B is Bn-dU.
  misc_feature (22): B is Bn-dU.
  misc_feature (23): B is Bn-dU.
  misc_feature (27): B is Bn-dU.
  misc_feature (30): B is Bn-dU.
  misc_feature (34): B is Bn-dU.
  misc_feature (39): B is Bn-dU.
  misc_feature (41): B is Bn-dU.

SEQ ID NO: 11 - DNA, 41 bp, Artificial Sequence; identical to SEQ ID NO: 1
  AMe 7
  misc_feature (4): B is Bn-dU.
  misc_feature (5): B is Bn-dU.
  misc_feature (12): B is Bn-dU.
  misc_feature (14): B is Bn-dU.
  misc_feature (18): B is Bn-dU.
  misc_feature (20): A is a base in which the -OH group at the 2nd carbon position in the nucleotide is substituted with methoxy.
  misc_feature (21): B is Bn-dU.
  misc_feature (22): B is Bn-dU.
  misc_feature (23): B is Bn-dU.
  misc_feature (27): B is Bn-dU.
  misc_feature (30): B is Bn-dU.
  misc_feature (34): B is Bn-dU.
  misc_feature (39): B is Bn-dU.
  misc_feature (41): B is Bn-dU.

SEQ ID NO: 12 - DNA, 41 bp, Artificial Sequence; identical to SEQ ID NO: 1
  AMe 8
  misc_feature (4): B is Bn-dU.
  misc_feature (5): B is Bn-dU.
  misc_feature (12): B is Bn-dU.
  misc_feature (14): B is Bn-dU.
  misc_feature (18): B is Bn-dU.
  misc_feature (21): B is Bn-dU.
  misc_feature (22): B is Bn-dU.
  misc_feature (23): B is Bn-dU.
  misc_feature (27): B is Bn-dU.
  misc_feature (30): B is Bn-dU.
  misc_feature (34): B is Bn-dU.
  misc_feature (37): A is a base in which the -OH group at the 2nd carbon position in the nucleotide is substituted with methoxy.
  misc_feature (39): B is Bn-dU.
  misc_feature (41): B is Bn-dU.

SEQ ID NO: 13 - DNA, 41 bp, Artificial Sequence; identical to SEQ ID NO: 1
  AMe 9
  misc_feature (4): B is Bn-dU.
  misc_feature (5): B is Bn-dU.
  misc_feature (12): B is Bn-dU.
  misc_feature (14): B is Bn-dU.
  misc_feature (18): B is Bn-dU.
  misc_feature (21): B is Bn-dU.
  misc_feature (22): B is Bn-dU.
  misc_feature (23): B is Bn-dU.
  misc_feature (27): B is Bn-dU.
  misc_feature (30): B is Bn-dU.
  misc_feature (34): B is Bn-dU.
  misc_feature (38): A is a base in which the -OH group at the 2nd carbon position in the nucleotide is substituted with methoxy.
  misc_feature (39): B is Bn-dU.
  misc_feature (41): B is Bn-dU.

SEQ ID NO: 14 - DNA, 41 bp, Artificial Sequence
  UMe 1
  misc_feature (4): U is a base in which the -OH group at the 2nd carbon position in the nucleotide is substituted with methoxy.
  misc_feature (5): B is Bn-dU.
  misc_feature (12): B is Bn-dU.
  misc_feature (14): B is Bn-dU.
  misc_feature (18): B is Bn-dU.
  misc_feature (21): B is Bn-dU.
  misc_feature (22): B is Bn-dU.
  misc_feature (23): B is Bn-dU.
  misc_feature (27): B is Bn-dU.
  misc_feature (30): B is Bn-dU.
  misc_feature (34): B is Bn-dU.
  misc_feature (39): B is Bn-dU.
  misc_feature (41): B is Bn-dU.
gaaubcaaaagbgbcggbgabbbgccbcgbcgcbccaabgb

SEQ ID NO: 15 - DNA, 41 bp, Artificial Sequence
  UMe 2
  misc_feature (4): B is Bn-dU.
  misc_feature (5): U is a base in which the -OH group at the 2nd carbon position in the nucleotide is substituted with methoxy.
  misc_feature (12): B is Bn-dU.
  misc_feature (14): B is Bn-dU.
  misc_feature (18): B is Bn-dU.
  misc_feature (21): B is Bn-dU.
  misc_feature (22): B is Bn-dU.
  misc_feature (23): B is Bn-dU.
  misc_feature (27): B is Bn-dU.
  misc_feature (30): B is Bn-dU.
  misc_feature (34): B is Bn-dU.
  misc_feature (39): B is Bn-dU.
  misc_feature (41): B is Bn-dU.
gaabucaaaagbgbcggbgabbbgccbcgbcgcbccaabgb

SEQ ID NO: 16 - DNA, 41 bp, Artificial Sequence
  UMe 3
  misc_feature (4): B is Bn-dU.
  misc_feature (5): B is Bn-dU.
  misc_feature (12): U is a base in which the -OH group at the 2nd carbon position in the nucleotide is substituted with methoxy.
  misc_feature (14): B is Bn-dU.
  misc_feature (18): B is Bn-dU.
  misc_feature (21): B is Bn-dU.
  misc_feature (22): B is Bn-dU.
  misc_feature (23): B is Bn-dU.
  misc_feature (27): B is Bn-dU.
  misc_feature (30): B is Bn-dU.
  misc_feature (34): B is Bn-dU.
  misc_feature (39): B is Bn-dU.
  misc_feature (41): B is Bn-dU.
gaabbcaaaagugbcggbgabbbgccbcgbcgcbccaabgb

SEQ ID NO: 17 - DNA, 41 bp, Artificial Sequence
  UMe 4
  misc_feature (4): B is Bn-dU.
  misc_feature (5): B is Bn-dU.
  misc_feature (12): B is Bn-dU.
  misc_feature (14): U is a base in which the -OH group at the 2nd carbon position in the nucleotide is substituted with methoxy.
  misc_feature (18): B is Bn-dU.
  misc_feature (21): B is Bn-dU.
  misc_feature (22): B is Bn-dU.
  misc_feature (23): B is Bn-dU.
  misc_feature (27): B is Bn-dU.
  misc_feature (30): B is Bn-dU.
  misc_feature (34): B is Bn-dU.
  misc_feature (39): B is Bn-dU.
  misc_feature (41): B is Bn-dU.
gaabbcaaaagbgucggbgabbbgccbcgbcgcbccaabgb

SEQ ID NO: 18 - DNA, 41 bp, Artificial Sequence
  UMe 5
  misc_feature (4): B is Bn-dU.
  misc_feature (5): B is Bn-dU.
  misc_feature (12): B is Bn-dU.
  misc_feature (14): B is Bn-dU.
  misc_feature (18): U is a base in which the -OH group at the 2nd carbon position in the nucleotide is substituted with methoxy.
  misc_feature (21): B is Bn-dU.
  misc_feature (22): B is Bn-dU.
  misc_feature (23): B is Bn-dU.
  misc_feature (27): B is Bn-dU.
  misc_feature (30): B is Bn-dU.
  misc_feature (34): B is Bn-dU.
  misc_feature (39): B is Bn-dU.
  misc_feature (41): B is Bn-dU.
gaabbcaaaagbgbcggugabbbgccbcgbcgcbccaabgb

SEQ ID NO: 19 - DNA, 41 bp, Artificial Sequence
  UMe 6
  misc_feature (4): B is Bn-dU.
  misc_feature (5): B is Bn-dU.
  misc_feature (12): B is Bn-dU.
  misc_feature (14): B is Bn-dU.
  misc_feature (18): B is Bn-dU.
  misc_feature (21): U is a base in which the -OH group at the 2nd carbon position in the nucleotide is substituted with methoxy.
  misc_feature (22): B is Bn-dU.
  misc_feature (23): B is Bn-dU.
  misc_feature (27): B is Bn-dU.
  misc_feature (30): B is Bn-dU.
  misc_feature (34): B is Bn-dU.
  misc_feature (39): B is Bn-dU.
  misc_feature (41): B is Bn-dU.
gaabbcaaaagbgbcggbgaubbgccbcgbcgcbccaabgb

SEQ ID NO: 20 - DNA, 41 bp, Artificial Sequence
  UMe 7
  misc_feature (4): B is Bn-dU.
  misc_feature (5): B is Bn-dU.
  misc_feature (12): B is Bn-dU.
  misc_feature (14): B is Bn-dU.
  misc_feature (18): B is Bn-dU.
  misc_feature (21): B is Bn-dU.
  misc_feature (22): U is a base in which the -OH group at the 2nd carbon position in the nucleotide is substituted with methoxy.
  misc_feature (23): B is Bn-dU.
  misc_feature (27): B is Bn-dU.
  misc_feature (30): B is Bn-dU.
  misc_feature (34): B is Bn-dU.
  misc_feature (39): B is Bn-dU.
  misc_feature (41): B is Bn-dU.
gaabbcaaaagbgbcggbgabubgccbcgbcgcbccaabgb

SEQ ID NO: 21 - DNA, 41 bp, Artificial Sequence
  UMe 8
  misc_feature (4): B is Bn-dU.
  misc_feature (5): B is Bn-dU.
  misc_feature (12): B is Bn-dU.
  misc_feature (14): B is Bn-dU.
  misc_feature (18): B is Bn-dU.
  misc_feature (21): B is Bn-dU.
  misc_feature (22): B is Bn-dU.
  misc_feature (23): U is a base in which the -OH group at the 2nd carbon position in the nucleotide is substituted with methoxy.
  misc_feature (27): B is Bn-dU.
  misc_feature (30): B is Bn-dU.
  misc_feature (34): B is Bn-dU.
  misc_feature (39): B is Bn-dU.
  misc_feature (41): B is Bn-dU.
gaabbcaaaagbgbcggbgabbugccbcgbcgcbccaabgb

SEQ ID NO: 22 - DNA, 41 bp, Artificial Sequence
  UMe 9
  misc_feature (4): B is Bn-dU.
  misc_feature (5): B is Bn-dU.
  misc_feature (12): B is Bn-dU.
  misc_feature (14): B is Bn-dU.
  misc_feature (18): B is Bn-dU.
  misc_feature (21): B is Bn-dU.
  misc_feature (22): B is Bn-dU.
  misc_feature (23): B is Bn-dU.
  misc_feature (27): U is a base in which the -OH group at the 2nd carbon position in the nucleotide is substituted with methoxy.
  misc_feature (30): B is Bn-dU.
  misc_feature (34): B is Bn-dU.
  misc_feature (39): B is Bn-dU.
  misc_feature (41): B is Bn-dU.
gaabbcaaaagbgbcggbgabbbgccucgbcgcbccaabgb

SEQ ID NO: 23 - DNA, 41 bp, Artificial Sequence
  UMe 10
  misc_feature (4): B is Bn-dU.
  misc_feature (5): B is Bn-dU.
  misc_feature (12): B is Bn-dU.
  misc_feature (14): B is Bn-dU.
  misc_feature (18): B is Bn-dU.
  misc_feature (21): B is Bn-dU.
  misc_feature (22): B is Bn-dU.
  misc_feature (23): B is Bn-dU.
  misc_feature (27): B is Bn-dU.
  misc_feature (30): U is a base in which the -OH group at the 2nd carbon position in the nucleotide is substituted with methoxy.
  misc_feature (34): B is Bn-dU.
  misc_feature (39): B is Bn-dU.
  misc_feature (41): B is Bn-dU.
gaabbcaaaagbgbcggbgabbbgccbcgucgcbccaabgb

SEQ ID NO: 24 - DNA, 41 bp, Artificial Sequence
  UMe 11
  misc_feature (4): B is Bn-dU.
  misc_feature (5): B is Bn-dU.
  misc_feature (12): B is Bn-dU.
  misc_feature (14): B is Bn-dU.
  misc_feature (18): B is Bn-dU.
  misc_feature (21): B is Bn-dU.
  misc_feature (22): B is Bn-dU.
  misc_feature (23): B is Bn-dU.
  misc_feature (27): B is Bn-dU.
  misc_feature (30): B is Bn-dU.
  misc_feature (34): U is a base in which the -OH group at the 2nd carbon position in the nucleotide is substituted with methoxy.
  misc_feature (39): B is Bn-dU.
  misc_feature (41): B is Bn-dU.
gaabbcaaaagbgbcggbgabbbgccbcgbcgcuccaabgb

SEQ ID NO: 25 - DNA, 41 bp, Artificial Sequence
  UMe 12
  misc_feature (4): B is Bn-dU.
  misc_feature (5): B is Bn-dU.
  misc_feature (12): B is Bn-dU.
  misc_feature (14): B is Bn-dU.
  misc_feature (18): B is Bn-dU.
  misc_feature (21): B is Bn-dU.
  misc_feature (22): B is Bn-dU.
  misc_feature (23): B is Bn-dU.
  misc_feature (27): B is Bn-dU.
  misc_feature (30): B is Bn-dU.
  misc_feature (34): B is Bn-dU.
  misc_feature (39): U is a base in which the -OH group at the 2nd carbon position in the nucleotide is substituted with methoxy.
  misc_feature (41): B is Bn-dU.
gaabbcaaaagbgbcggbgabbbgccbcgbcgcbccaaugb

SEQ ID NO: 26 - DNA, 41 bp, Artificial Sequence
  UMe 13
  misc_feature (4): B is Bn-dU.
  misc_feature (5): B is Bn-dU.
  misc_feature (12): B is Bn-dU.
  misc_feature (14): B is Bn-dU.
  misc_feature (18): B is Bn-dU.
  misc_feature (21): B is Bn-dU.
  misc_feature (22): B is Bn-dU.
  misc_feature (23): B is Bn-dU.
  misc_feature (27): B is Bn-dU.
  misc_feature (30): B is Bn-dU.
  misc_feature (34): B is Bn-dU.
  misc_feature (39): B is Bn-dU.
  misc_feature (41): U is a base in which the -OH group at the 2nd carbon position in the nucleotide is substituted with methoxy.
gaabbcaaaagbgbcggbgabbbgccbcgbcgcbccaabgu

SEQ ID NO: 27 - DNA, 41 bp, Artificial Sequence; identical to SEQ ID NO: 1
  GMe 1
  misc_feature (1): G is a base in which the -OH group at the 2nd carbon position in the nucleotide is substituted with methoxy.
  misc_feature (4): B is Bn-dU.
  misc_feature (5): B is Bn-dU.
  misc_feature (12): B is Bn-dU.
  misc_feature (14): B is Bn-dU.
  misc_feature (18): B is Bn-dU.
  misc_feature (21): B is Bn-dU.
  misc_feature (22): B is Bn-dU.
  misc_feature (23): B is Bn-dU.
  misc_feature (27): B is Bn-dU.
  misc_feature (30): B is Bn-dU.
  misc_feature (34): B is Bn-dU.
  misc_feature (39): B is Bn-dU.
  misc_feature (41): B is Bn-dU.

SEQ ID NO: 28 - DNA, 41 bp, Artificial Sequence; identical to SEQ ID NO: 1
  GMe 2
  misc_feature (4): B is Bn-dU.
  misc_feature (5): B is Bn-dU.
  misc_feature (11): G is a base in which the -OH group at the 2nd carbon position in the nucleotide is substituted with methoxy.
  misc_feature (12): B is Bn-dU.
  misc_feature (14): B is Bn-dU.
  misc_feature (18): B is Bn-dU.
  misc_feature (21): B is Bn-dU.
  misc_feature (22): B is Bn-dU.
  misc_feature (23): B is Bn-dU.
  misc_feature (27): B is Bn-dU.
  misc_feature (30): B is Bn-dU.
  misc_feature (34): B is Bn-dU.
  misc_feature (39): B is Bn-dU.
  misc_feature (41): B is Bn-dU.

SEQ ID NO: 29 - DNA, 41 bp, Artificial Sequence; identical to SEQ ID NO: 1
  GMe 3
  misc_feature (4): B is Bn-dU.
  misc_feature (5): B is Bn-dU.
  misc_feature (12): B is Bn-dU.
  misc_feature (13): G is a base in which the -OH group at the 2nd carbon position in the nucleotide is substituted with methoxy.
  misc_feature (14): B is Bn-dU.
  misc_feature (18): B is Bn-dU.
  misc_feature (21): B is Bn-dU.
  misc_feature (22): B is Bn-dU.
  misc_feature (23): B is Bn-dU.
  misc_feature (27): B is Bn-dU.
  misc_feature (30): B is Bn-dU.
  misc_feature (34): B is Bn-dU.
  misc_feature (39): B is Bn-dU.
  misc_feature (41): B is Bn-dU.

SEQ ID NO: 30 - DNA, 41 bp, Artificial Sequence; identical to SEQ ID NO: 1
  GMe 4
  misc_feature (4): B is Bn-dU.
  misc_feature (5): B is Bn-dU.
  misc_feature (12): B is Bn-dU.
  misc_feature (14): B is Bn-dU.
  misc_feature (16): G is a base in which the -OH group at the 2nd carbon position in the nucleotide is substituted with methoxy.
  misc_feature (18): B is Bn-dU.
  misc_feature (21): B is Bn-dU.
  misc_feature (22): B is Bn-dU.
  misc_feature (23): B is Bn-dU.
  misc_feature (27): B is Bn-dU.
  misc_feature (30): B is Bn-dU.
  misc_feature (34): B is Bn-dU.
  misc_feature (39): B is Bn-dU.
  misc_feature (41): B is Bn-dU.

SEQ ID NO: 31 - DNA, 41 bp, Artificial Sequence; identical to SEQ ID NO: 1
  GMe 5
  misc_feature (4): B is Bn-dU.
  misc_feature (5): B is Bn-dU.
  misc_feature (12): B is Bn-dU.
  misc_feature (14): B is Bn-dU.
  misc_feature (17): G is a base in which the -OH group at the 2nd carbon position in the nucleotide is substituted with methoxy.
  misc_feature (18): B is Bn-dU.
  misc_feature (21): B is Bn-dU.
  misc_feature (22): B is Bn-dU.
  misc_feature (23): B is Bn-dU.
  misc_feature (27): B is Bn-dU.
  misc_feature (30): B is Bn-dU.
  misc_feature (34): B is Bn-dU.
  misc_feature (39): B is Bn-dU.
  misc_feature (41): B is Bn-dU.

SEQ ID NO: 32 - DNA, 41 bp, Artificial Sequence; identical to SEQ ID NO: 1
  GMe 6
  misc_feature (4): B is Bn-dU.
  misc_feature (5): B is Bn-dU.
  misc_feature (12): B is Bn-dU.
  misc_feature (14): B is Bn-dU.
  misc_feature (18): B is Bn-dU.
  misc_feature (19): G is a base in which the -OH group at the 2nd carbon position in the nucleotide is substituted with methoxy.
  misc_feature (21): B is Bn-dU.
  misc_feature (22): B is Bn-dU.
  misc_feature (23): B is Bn-dU.
  misc_feature (27): B is Bn-dU.
  misc_feature (30): B is Bn-dU.
  misc_feature (34): B is Bn-dU.
  misc_feature (39): B is Bn-dU.
  misc_feature (41): B is Bn-dU.

SEQ ID NO: 33 - DNA, 41 bp, Artificial Sequence; identical to SEQ ID NO: 1
  GMe 7
  misc_feature (4): B is Bn-dU.
  misc_feature (5): B is Bn-dU.
  misc_feature (12): B is Bn-dU.
  misc_feature (14): B is Bn-dU.
  misc_feature (18): B is Bn-dU.
  misc_feature (21): B is Bn-dU.
  misc_feature (22): B is Bn-dU.
  misc_feature (23): B is Bn-dU.
  misc_feature (24): G is a base in which the -OH group at the 2nd carbon position in the nucleotide is substituted with methoxy.
  misc_feature (27): B is Bn-dU.
  misc_feature (30): B is Bn-dU.
  misc_feature (34): B is Bn-dU.
  misc_feature (39): B is Bn-dU.
  misc_feature (41): B is Bn-dU.

SEQ ID NO: 34 - DNA, 41 bp, Artificial Sequence; identical to SEQ ID NO: 1
  GMe 8
  misc_feature (4): B is Bn-dU.
  misc_feature (5): B is Bn-dU.
  misc_feature (12): B is Bn-dU.
  misc_feature (14): B is Bn-dU.
  misc_feature (18): B is Bn-dU.
  misc_feature (21): B is Bn-dU.
  misc_feature (22): B is Bn-dU.
  misc_feature (23): B is Bn-dU.
  misc_feature (27): B is Bn-dU.
  misc_feature (29): G is a base in which the -OH group at the 2nd carbon position in the nucleotide is substituted with methoxy.
  misc_feature (30): B is Bn-dU.
  misc_feature (34): B is Bn-dU.
  misc_feature (39): B is Bn-dU.
  misc_feature (41): B is Bn-dU.

SEQ ID NO: 35 - DNA, 41 bp, Artificial Sequence; identical to SEQ ID NO: 1
  GMe 9
  misc_feature (4): B is Bn-dU.
  misc_feature (5): B is Bn-dU.
  misc_feature (12): B is Bn-dU.
  misc_feature (14): B is Bn-dU.
  misc_feature (18): B is Bn-dU.
  misc_feature (21): B is Bn-dU.
  misc_feature (22): B is Bn-dU.
  misc_feature (23): B is Bn-dU.
  misc_feature (27): B is Bn-dU.
  misc_feature (30): B is Bn-dU.
  misc_feature (32): G is a base in which the -OH group at the 2nd carbon position in the nucleotide is substituted with methoxy.
  misc_feature (34): B is Bn-dU.
  misc_feature (39): B is Bn-dU.
  misc_feature (41): B is Bn-dU.

SEQ ID NO: 36 - DNA, 41 bp, Artificial Sequence; identical to SEQ ID NO: 1
  GMe 10
  misc_feature (4): B is Bn-dU.
  misc_feature (5): B is Bn-dU.
  misc_feature (12): B is Bn-dU.
  misc_feature (14): B is Bn-dU.
  misc_feature (18): B is Bn-dU.
  misc_feature (21): B is Bn-dU.
  misc_feature (22): B is Bn-dU.
  misc_feature (23): B is Bn-dU.
  misc_feature (27): B is Bn-dU.
  misc_feature (30): B is Bn-dU.
  misc_feature (34): B is Bn-dU.
  misc_feature (39): B is Bn-dU.
  misc_feature (40): G is a base in which the -OH group at the 2nd carbon position in the nucleotide is substituted with methoxy.
  misc_feature (41): B is Bn-dU.

SEQ ID NO: 37 - DNA, 41 bp, Artificial Sequence; identical to SEQ ID NO: 1
  CMe 1
  misc_feature (4): B is Bn-dU.
  misc_feature (5): B is Bn-dU.
  misc_feature (6): C is a base in which the -OH group at the 2nd carbon position in the nucleotide is substituted with methoxy.
  misc_feature (12): B is Bn-dU.
  misc_feature (14): B is Bn-dU.
  misc_feature (18): B is Bn-dU.
  misc_feature (21): B is Bn-dU.
  misc_feature (22): B is Bn-dU.
  misc_feature (23): B is Bn-dU.
  misc_feature (27): B is Bn-dU.
  misc_feature (30): B is Bn-dU.
  misc_feature (34): B is Bn-dU.
  misc_feature (39): B is Bn-dU.
  misc_feature (41): B is Bn-dU.

SEQ ID NO: 38 - DNA, 41 bp, Artificial Sequence; identical to SEQ ID NO: 1
  CMe 2
  misc_feature (4): B is Bn-dU.
  misc_feature (5): B is Bn-dU.
  misc_feature (12): B is Bn-dU.
  misc_feature (14): B is Bn-dU.
  misc_feature (15): C is a base in which the -OH group at the 2nd carbon position in the nucleotide is substituted with methoxy.
  misc_feature (18): B is Bn-dU.
  misc_feature (21): B is Bn-dU.
  misc_feature (22): B is Bn-dU.
  misc_feature (23): B is Bn-dU.
  misc_feature (27): B is Bn-dU.
  misc_feature (30): B is Bn-dU.
  misc_feature (34): B is Bn-dU.
  misc_feature (39): B is Bn-dU.
  misc_feature (41): B is Bn-dU.

SEQ ID NO: 39 - DNA, 41 bp, Artificial Sequence; identical to SEQ ID NO: 1
  CMe 3
  misc_feature (4): B is Bn-dU.
  misc_feature (5): B is Bn-dU.
  misc_feature (12): B is Bn-dU.
  misc_feature (14): B is Bn-dU.
  misc_feature (18): B is Bn-dU.
  misc_feature (21): B is Bn-dU.
  misc_feature (22): B is Bn-dU.
  misc_feature (23): B is Bn-dU.
  misc_feature (25): C is a base in which the -OH group at the 2nd carbon position in the nucleotide is substituted with methoxy.
  misc_feature (27): B is Bn-dU.
  misc_feature (30): B is Bn-dU.
  misc_feature (34): B is Bn-dU.
  misc_feature (39): B is Bn-dU.
  misc_feature (41): B is Bn-dU.

SEQ ID NO: 40 - DNA, 41 bp, Artificial Sequence; identical to SEQ ID NO: 1
  CMe 4
  misc_feature (4): B is Bn-dU.
  misc_feature (5): B is Bn-dU.
  misc_feature (12): B is Bn-dU.
  misc_feature (14): B is Bn-dU.
  misc_feature (18): B is Bn-dU.
  misc_feature (21): B is Bn-dU.
  misc_feature (22): B is Bn-dU.
  misc_feature (23): B is Bn-dU.
  misc_feature (26): C is a base in which the -OH group at the 2nd carbon position in the nucleotide is substituted with methoxy.
  misc_feature (27): B is Bn-dU.
  misc_feature (30): B is Bn-dU.
  misc_feature (34): B is Bn-dU.
  misc_feature (39): B is Bn-dU.
  misc_feature (41): B is Bn-dU.

SEQ ID NO: 41 - DNA, 41 bp, Artificial Sequence; identical to SEQ ID NO: 1
  CMe 5
  misc_feature (4): B is Bn-dU.
  misc_feature (5): B is Bn-dU.
  misc_feature (12): B is Bn-dU.
  misc_feature (14): B is Bn-dU.
  misc_feature (18): B is Bn-dU.
  misc_feature (21): B is Bn-dU.
  misc_feature (22): B is Bn-dU.
  misc_feature (23): B is Bn-dU.
  misc_feature (27): B is Bn-dU.
  misc_feature (28): C is a base in which the -OH group at the 2nd carbon position in the nucleotide is substituted with methoxy.
  misc_feature (30): B is Bn-dU.
  misc_feature (34): B is Bn-dU.
  misc_feature (39): B is Bn-dU.
  misc_feature (41): B is Bn-dU.

SEQ ID NO: 42 - DNA, 41 bp, Artificial Sequence; identical to SEQ ID NO: 1
  CMe 6
  misc_feature (4): B is Bn-dU.
  misc_feature (5): B is Bn-dU.
  misc_feature (12): B is Bn-dU.
  misc_feature (14): B is Bn-dU.
  misc_feature (18): B is Bn-dU.
  misc_feature (21): B is Bn-dU.
  misc_feature (22): B is Bn-dU.
  misc_feature (23): B is Bn-dU.
  misc_feature (27): B is Bn-dU.
  misc_feature (30): B is Bn-dU.
  misc_feature (31): C is a base in which the -OH group at the 2nd carbon position in the nucleotide is substituted with methoxy.
  misc_feature (34): B is Bn-dU.
  misc_feature (39): B is Bn-dU.
  misc_feature (41): B is Bn-dU.

SEQ ID NO: 43 - DNA, 41 bp, Artificial Sequence; identical to SEQ ID NO: 1
  CMe 7
  misc_feature (4): B is Bn-dU.
  misc_feature (5): B is Bn-dU.
  misc_feature (12): B is Bn-dU.
  misc_feature (14): B is Bn-dU.
  misc_feature (18): B is Bn-dU.
  misc_feature (21): B is Bn-dU.
  misc_feature (22): B is Bn-dU.
  misc_feature (23): B is Bn-dU.
  misc_feature (27): B is Bn-dU.
  misc_feature (30): B is Bn-dU.
  misc_feature (33): C is a base in which the -OH group at the 2nd carbon position in the nucleotide is substituted with methoxy.
  misc_feature (34): B is Bn-dU.
  misc_feature (39): B is Bn-dU.
  misc_feature (41): B is Bn-dU.

SEQ ID NO: 44 - DNA, 41 bp, Artificial Sequence; identical to SEQ ID NO: 1
  CMe 8
  misc_feature (4): B is Bn-dU.
  misc_feature (5): B is Bn-dU.
  misc_feature (12): B is Bn-dU.
  misc_feature (14): B is Bn-dU.
  misc_feature (18): B is Bn-dU.
  misc_feature (21): B is Bn-dU.
  misc_feature (22): B is Bn-dU.
  misc_feature (23): B is Bn-dU.
  misc_feature (27): B is Bn-dU.
  misc_feature (30): B is Bn-dU.
  misc_feature (34): B is Bn-dU.
  misc_feature (35): C is a base in which the -OH group at the 2nd carbon position in the nucleotide is substituted with methoxy.
  misc_feature (39): B is Bn-dU.
  misc_feature (41): B is Bn-dU.

SEQ ID NO: 45 - DNA, 41 bp, Artificial Sequence; identical to SEQ ID NO: 1
  CMe 9
  misc_feature (4): B is Bn-dU.
  misc_feature (5): B is Bn-dU.
  misc_feature (12): B is Bn-dU.
  misc_feature (14): B is Bn-dU.
  misc_feature (18): B is Bn-dU.
  misc_feature (21): B is Bn-dU.
  misc_feature (22): B is Bn-dU.
  misc_feature (23): B is Bn-dU.
  misc_feature (27): B is Bn-dU.
  misc_feature (30): B is Bn-dU.
  misc_feature (34): B is Bn-dU.
  misc_feature (36): C is a base in which the -OH group at the 2nd carbon position in the nucleotide is substituted with methoxy.
  misc_feature (39): B is Bn-dU.
  misc_feature (41): B is Bn-dU.

SEQ ID NO: 46 - DNA, 41 bp, Artificial Sequence; identical to SEQ ID NO: 1
  TfR 41 mer_combi 1
  misc_feature (4): B is Bn-dU.
  misc_feature (5): B is Bn-dU.
  misc_feature (6): C is a base in which the -OH group at the 2nd carbon position in the nucleotide is substituted with methoxy.
  misc_feature (11): G is a base in which the -OH group at the 2nd carbon position in the nucleotide is substituted with methoxy.
  misc_feature (12): B is Bn-dU.
  misc_feature (14): B is Bn-dU.
  misc_feature (16): G is a base in which the -OH group at the 2nd carbon position in the nucleotide is substituted with methoxy.
  misc_feature (18): B is Bn-dU.
  misc_feature (21): B is Bn-dU.
  misc_feature (22): B is Bn-dU.
  misc_feature (23): B is Bn-dU.
  misc_feature (27): B is Bn-dU.
  misc_feature (29): G is a base in which the -OH group at the 2nd carbon position in the nucleotide is substituted with methoxy.
  misc_feature (30): B is Bn-dU.
  misc_feature (34): B is Bn-dU.
  misc_feature (35): C is a base in which the -OH group at the 2nd carbon position in the nucleotide is substituted with methoxy.
  misc_feature (36): C is a base in which the -OH group at the 2nd carbon position in the nucleotide is substituted with methoxy.
  misc_feature (39): B is Bn-dU.
  misc_feature (41): B is Bn-dU.

SEQ ID NO: 47 - DNA, 41 bp, Artificial Sequence; identical to SEQ ID NO: 1
  TfR 41 mer_combi 2
  misc_feature (4): B is Bn-dU.
  misc_feature (5): B is Bn-dU.
  misc_feature (6): C is a base in which the -OH group at the 2nd carbon position in the nucleotide is substituted with methoxy.
  misc_feature (12): B is Bn-dU.
  misc_feature (14): B is Bn-dU.
  misc_feature (18): B is Bn-dU.
  misc_feature (21): B is Bn-dU.
  misc_feature (22): B is Bn-dU.
  misc_feature (23): B is Bn-dU.
  misc_feature (27): B is Bn-dU.
  misc_feature (30): B is Bn-dU.
  misc_feature (34): B is Bn-dU.
  misc_feature (35): C is a base in which the -OH group at the 2nd carbon position in the nucleotide is substituted with methoxy.
  misc_feature (36): C is a base in which the -OH group at the 2nd carbon position in the nucleotide is substituted with methoxy.
  misc_feature (39): B is Bn-dU.
  misc_feature (41): B is Bn-dU.

SEQ ID NO: 48 - DNA, 41 bp, Artificial Sequence; identical to SEQ ID NO: 1
  TfR 41 mer_combi 3
  misc_feature (4): B is Bn-dU.
  misc_feature (5): B is Bn-dU.
  misc_feature (11): G is a base in which the -OH group at the 2nd carbon position in the nucleotide is substituted with methoxy.
  misc_feature (12): B is Bn-dU.
  misc_feature (14): B is Bn-dU.
  misc_feature (18): B is Bn-dU.
  misc_feature (21): B is Bn-dU.
  misc_feature (22): B is Bn-dU.
  misc_feature (23): B is Bn-dU.
  misc_feature (27): B is Bn-dU.
  misc_feature (29): G is a base in which the -OH group at the 2nd carbon position in the nucleotide is substituted with methoxy.
  misc_feature (30): B is Bn-dU.
  misc_feature (34): B is Bn-dU.
  misc_feature (39): B is Bn-dU.
  misc_feature (41): B is Bn-dU.
  misc_feature (16): G is a base in which the -OH group at the 2nd carbon position in the nucleotide is substituted with methoxy.

SEQ ID NO: 49 - DNA, 41 bp, Artificial Sequence; identical to SEQ ID NO: 20
  TfR 41 mer_combi 4
  misc_feature (4): B is Bn-dU.
  misc_feature (5): B is Bn-dU.
  misc_feature (12): B is Bn-dU.
  misc_feature (14): B is Bn-dU.
  misc_feature (16): G is a base in which the -OH group at the 2nd carbon position in the nucleotide is substituted with methoxy.
  misc_feature (18): B is Bn-dU.
  misc_feature (21): B is Bn-dU.
  misc_feature (22): U is a base in which the -OH group at the 2nd carbon position in the nucleotide is substituted with methoxy.
  misc_feature (23): B is Bn-dU.
  misc_feature (26): C is a base in which the -OH group at the 2nd carbon position in the nucleotide is substituted with methoxy.
  misc_feature (27): B is Bn-dU.
  misc_feature (29): G is a base in which the -OH group at the 2nd carbon position in the nucleotide is substituted with methoxy.
  misc_feature (30): B is Bn-dU.
  misc_feature (34): B is Bn-dU.
  misc_feature (35): C is a base in which the -OH group at the 2nd carbon position in the nucleotide is substituted with methoxy.
  misc_feature (36): C is a base in which the -OH group at the 2nd carbon position in the nucleotide is substituted with methoxy.
  misc_feature (39): B is Bn-dU.
  misc_feature (41): B is Bn-dU.

SEQ ID NO: 50 - DNA, 22 bp, Artificial Sequence
  forward primer
agaattcaaaagtgtcggtgat

SEQ ID NO: 51 - DNA, 22 bp, Artificial Sequence
  reverse primer
cgccaacattggagccacgagg

SEQ ID NO: 52 - DNA, 25 bp, Artificial Sequence
  General formula 1
agtgtcggtgatttgcctcgtcgct